European Patent Specification EP 3 977 848 B1, published September 25, 2024. Title: TRANSGENIC MOUSE MODEL OF MYELIN PATHOLOGIES. Applicant: Universidad Autónoma de Madrid. The sequence listing filed with the application follows.

SEQUENCE LISTING (7 sequences)

SEQ ID NO: 1 - DNA, 25 bp, Artificial sequence
  Artificial sequence
ggagcaagaggagggaaggaatggg

SEQ ID NO: 2 - DNA, 25 bp, Artificial sequence
  Artificial sequence
ccttccagaggactcagttcaatcc

SEQ ID NO: 3 - DNA, 20 bp, Artificial sequence
  Artificial sequence
cgctctagctgagcctctgt

SEQ ID NO: 4 - DNA, 20 bp, Artificial sequence
  Artificial sequence
tacagggtcttgtggggaaa

SEQ ID NO: 5 - DNA, 23 bp, Artificial sequence
  Artificial sequence
tgaaacaggatcatgttgtggag

SEQ ID NO: 6 - DNA, 20 bp, Artificial sequence
  Artificial sequence
caggaggagtccaagaagac

SEQ ID NO: 7 - DNA, 23 bp, Artifical sequence
  Artificial sequence
ataaaccctcttgcagttgcatc